European Patent Application EP 4 112 635 A1, published January 4, 2023. Title: SARS-CoV-2的重组RBD蛋白及其制备方法. Applicant: 深圳市亚辉龙生物科技股份有限公司. The sequence listing filed with the application follows.

SEQUENCE LISTING (5 sequences)

SEQ ID NO: 1 - protein, 201 aa, artificial sequence
NITNLCPFGEVFNATRFASVYAWNRKRISNCVADYSVLYNSASFSTFKCYGVSPTKLNDLCFTNVYADSFVIRGDEVRQIAPGQTGKIADYNYKLPDDFTGCVIAWNSNNLDSKVGGNYNYLYRLFRKSNLKPFERDISTEIYQAGSTPCNGVEGFNCYFPLQSYGFQPTNGVGYQPYRVVVLSFELLHAPATVCGPKKST

SEQ ID NO: 2 - protein, 23 aa, artificial sequence
ELWLVLVAVGAGLLLLGLIILLL

SEQ ID NO: 3 - protein, 16 aa, artificial sequence
WGQGGTHGQWNKPSKP

SEQ ID NO: 4 - protein, 16 aa, artificial sequence
MFVFLVLLPLVSSQCV

SEQ ID NO: 5 - DNA, 771 bp, artificial sequence
atgtttgtttttcttgttttattgccactagtctctagtcagtgtgttaatattacaaacttgtgcccttttggtgaagtttttaacgccaccagatttgcatctgtttatgcttggaacaggaagagaatcagcaactgtgttgctgattattctgtcctatataattccgcatcattttccacttttaagtgttatggagtgtctcctactaaattaaatgatctctgctttactaatgtctatgcagattcatttgtaattagaggtgatgaagtcagacaaatcgctccagggcaaactggaaagattgctgattataattataaattaccagatgattttacaggctgcgttatagcttggaattctaacaatcttgattctaaggttggtggtaattataattacctgtatagattgtttaggaagtctaatctcaaaccttttgagagagatatttcaactgaaatctatcaggccggtagcacaccttgtaatggtgttgaaggttttaattgttactttcctttacaatcatatggtttccaacccactaatggtgttggttaccaaccatacagagtagtagtactttcttttgaacttctacatgcaccagcaactgtttgtggacctaaaaagtctactgagctgtggctggtgctggtggccgtgggcgctggactgctgctgctgggactgatcatcctgctgctgtggggtcaaggcggtacacatggtcaatggaacaagccttcgaagccgtga